European Patent Specification EP 3 655 436 B1, published October 15, 2025. Title: Serum albumin binding agents. Applicant: VIB VZW. The sequence listing filed with the application follows.

SEQUENCE LISTING (157 sequences)

SEQ ID NO: 1 - protein, 6 aa, Artificial Sequence
  CDR1 of SA1_S30K
KEYVMG

SEQ ID NO: 2 - protein, 13 aa, Artificial Sequence
  CDR2 of SA1_S30K
FVAAISWSAGNIY

SEQ ID NO: 3 - protein, 16 aa, Artificial Sequence
  CDR3 of SA1_S30K
AAGRYSAWYVAAYEYD

SEQ ID NO: 4 - skipped
  Full length SA1_S30K

SEQ ID NO: 5 - skipped
  Full length SA1

SEQ ID NO: 6 - skipped
  Full length VHH-GFP-SA1_S30K

SEQ ID NO: 7 - skipped

SEQ ID NO: 8 - skipped
  SA1_S30K_human1

SEQ ID NO: 9 - skipped
  SA1_S30K_human2

SEQ ID NO: 10 - skipped
  SA1_S30K_human3

SEQ ID NO: 11 - skipped
  SA1_S30K_human4

SEQ ID NO: 12-14 - skipped (3 entries)

SEQ ID NO: 15 - protein, 124 aa, Artificial Sequence
  humanized variant h5 of SA1_S30K
QVQLQESGGGLVQAGGSLRLSCAASGRNIKEYVMGWFRQAPGKEREFVAAISWSAGNIYYADSVKGRFTISRDNAKNTVYLQMNTLRPEDTAVYYCAAGRYSAWYVAAYEYDYWGQGTQVTVSS

SEQ ID NO: 16 - protein, 124 aa, Artificial Sequence
  humanized variant h6 of SA1_S30K
QVQLQESGGGLVQAGGSLRLSCAASGRNIKEYVMGWFRQAPGKEREFVAAISWSAGNIYYADSVKGRFTISRDNAKNTVHLQMNSLRPEDTAVYYCAAGRYSAWYVAAYEYDYWGQGTQVTVSS

SEQ ID NO: 17 - protein, 124 aa, Artificial Sequence
  humanized variant h7 of SA1_S30K
QVQLQESGGGLVQAGGSLRLSCAASGRNIKEYVMGWFRQAPGKEREFVAAISWSAGNIYYADSVKGRFTISRDNAKNTVYLQMNSLRPEDTAVYYCAAGRYSAWYVAAYEYDYWGQGTQVTVSS

SEQ ID NO: 18 - protein, 37 aa, Artificial Sequence
  FR3 from SA1_S30K
  misc_feature (15)..(16): Xaa can be any naturally occurring amino acid
YADSVKGRFTISRDXXKNTVHLQMNTLRPEDTAVYYC

SEQ ID NO: 19 - protein, 98 aa, Homo sapiens
EVQLVESGGGLVQPGGSLRLSCAASGFTFSSYWMSWVRQAPGKGLEWVANIKQDGSEKYYVDSVKGRFTISRDNAKNSLYLQMNSLRAEDTAVYYCAR

SEQ ID NO: 20 - protein, 98 aa, Homo sapiens; identical to SEQ ID NO: 19

SEQ ID NO: 21 - protein, 98 aa, Homo sapiens; identical to SEQ ID NO: 19

SEQ ID NO: 22 - protein, 99 aa, Homo sapiens
EVQLVESGGGLVQPGRSLRLSCAASGFTFDDYAMHWVRQAPGKGLEWVSGISWNSGSIGYADSVKGRFTISRDNAKNSLYLQMNSLRAEDTALYYCAKD

SEQ ID NO: 23 - protein, 99 aa, Homo sapiens
EVQLVESGGGLVQPGRSLRLSCAASGFTSDDYAMHWVRQAPGKGLEWVSGISWNSGSIGYADSVKGRFTISRDNAKNSLYLQMNSLRAEDTALYYCAKD

SEQ ID NO: 24 - protein, 99 aa, Homo sapiens
EVQLVESGGGLVQPGRSLRLSCAASGFTFDDYAMHWVRQAPGKGLEWVSGISWNSGSIGYADSVKGRFTISRDNAKNSLYLQMNSLRAEDMALYYCAKD

SEQ ID NO: 25 - protein, 98 aa, Homo sapiens
QVQLVESGGGLVKPGGSLRLSCAASGFTFSDYYMSWIRQAPGKGLEWVSYISSSGSTIYYADSVKGRFTISRDNAKNSLYLQMNSLRAEDTAVYYCAR

SEQ ID NO: 26 - protein, 98 aa, Homo sapiens
QVQLLESGGGLVKPGGSLRLSCAASGFTFSDYYMSWIRQAPGKGLEWVSYISSSSSYTNYADSVKGRFTISRDNAKNSLYLQMNSLRAEDTAVYYCAR

SEQ ID NO: 27 - protein, 98 aa, Homo sapiens; identical to SEQ ID NO: 25

SEQ ID NO: 28 - protein, 98 aa, Homo sapiens
QVQLVESGGGLVKPGGSLRLSCAASGFTFSDYYMSWIRQAPGKGLEWVSYISSSSSYTNYADSVKGRFTISRDNAKNSLYLQMNSLRAEDTAVYYCAR

SEQ ID NO: 29 - protein, 98 aa, Homo sapiens; identical to SEQ ID NO: 28

SEQ ID NO: 30 - protein, 97 aa, Homo sapiens
EVQLVESGGGLVQPGGSLRLSCAASGFTFSSYDMHWVRQATGKGLEWVSAIGTAGDTYYPGSVKGRFTISRENAKNSLYLQMNSLRAGDTAVYYCAR

SEQ ID NO: 31 - protein, 97 aa, Homo sapiens
EVHLVESGGGLVQPGGALRLSCAASGFTFSNYDMHWVRQATGKGLEWVSANGTAGDTYYPGSVKGRFTISRENAKNSLYLQMNSLRAGDTAVYYCAR

SEQ ID NO: 32 - protein, 97 aa, Homo sapiens
EVQLVESGGGLVQPGGSLRLSCAACGFTFSSYDMHWVRQATGKGLEWVSAIGTAGDTYYPGSVKGQFTISRENAKNSLYLQMNSLRAGDTAVYYCAR

SEQ ID NO: 33 - protein, 97 aa, Homo sapiens; identical to SEQ ID NO: 30

SEQ ID NO: 34 - protein, 97 aa, Homo sapiens
EVQLVESGGGLVQPGGSLRLSCAASGFTFSSYDMHWVRQATGKGLEWVSAIGTAGDPYYPGSVKGRFTISRENAKNSLYLQMNSLRAGDTAVYYCAR

SEQ ID NO: 35 - protein, 100 aa, Homo sapiens
EVQLVESGGGLVKPGGSLRLSCAASGFTFSNAWMSWVRQAPGKGLEWVGRIKSKTDGGTTDYAAPVKGRFTISRDDSKNTLYLQMNSLKTEDTAVYYCTT

SEQ ID NO: 36 - protein, 100 aa, Homo sapiens
EVQLVESGGALVKPGGSLRLSCAASGFTFSNAWMSWVRQAPGKGLEWVGRIKSKTDGGTTDYAAPVKGRFTISRDDSKNTLYLQMNSLKTEDTAVYYCTT

SEQ ID NO: 37 - protein, 100 aa, Homo sapiens
EVQLVESAGALVQPGGSLRLSCAASGFTCSNAWMSWVRQAPGKGLEWVGRIKSKANGGTTDYAAPVKGRFTISRVDSKNTLYLQMNSLKTEDTAVYYCTT

SEQ ID NO: 38 - protein, 100 aa, Homo sapiens
EVQLVESGGGLVKPGGSLRLSCAASGFTFSNAWMSWVRQAPGKGLEWVGRIESKTDGGTTDYAAPVKGRFTISRDDSKNTLYLQMNSLKTEDTAVYYCTT

SEQ ID NO: 39 - protein, 100 aa, Homo sapiens; identical to SEQ ID NO: 35

SEQ ID NO: 40 - protein, 100 aa, Homo sapiens
EVQLVESGGGLVKPGGSLRLSCAASGFTFSNAWMSWVRQAPGKGLEWVGRIKSKTDGGTTNYAAPVKGRFTISRDDSKNTLYLQMNSLKTEDTAVYYCTT

SEQ ID NO: 41 - protein, 100 aa, Homo sapiens
EVQLVESGGGLVKPGGSLRLSCAASGFTFSNAWMNWVRQAPGKGLEWVGRIKSKTDGGTTDYAAPVKGRFTISRDDSKNTLYLQMNSLKTEDTAVYYCTT

SEQ ID NO: 42 - protein, 100 aa, Homo sapiens
EVQLVESAGGLVQPGGSLRLSCAASGFTCSNAWMSWVRQAPGKGLEWVGCIKSKANGGTTDYAAPVKGRFTISRDDSKNTLYLQMISLKTEDTAVYYCTT

SEQ ID NO: 43 - protein, 98 aa, Homo sapiens
EVQLVESGGGLVQPGGSLRLSCAASGFTFSNSDMNWARKAPGKGLEWVSGVSWNGSRTHYVDSVKRRFIISRDNSRNSLYLQKNRRRAEDMAVYYCVR

SEQ ID NO: 44 - protein, 98 aa, Homo sapiens; identical to SEQ ID NO: 43

SEQ ID NO: 45 - protein, 98 aa, Homo sapiens
TVQLVESGGGLVEPGGSLRLSCAASGFTFSNSDMNWVRQAPGKGLEWVSGVSWNGSRTHYADSVKGRFIISRDNSRNFLYQQMNSLRPEDMAVYYCVR

SEQ ID NO: 46 - protein, 98 aa, Homo sapiens
EVQLVESGGGVVRPGGSLRLSCAASGFTFDDYGMSWVRQAPGKGLEWVSGINWNGGSTGYADSVKGRFTISRDNAKNSLYLQMNSLRAEDTALYHCAR

SEQ ID NO: 47 - protein, 98 aa, Homo sapiens
EVQLVESGGGVVRPGGSLRLSFAASGFTFDDYGMSWVRQAPGKGLEWVSGINWNGGSTGYADSVKGRFTISRDNAKNSLYLQMNSLRAEDTALYHCAR

SEQ ID NO: 48 - protein, 98 aa, Homo sapiens
EVQLVESGGGLVKPGGSLRLSCAASGFTFSSYSMNWVRQAPGKGLEWVSSISSSSSYIYYADSVKGRFTISRDNAKNSLYLQMNSLRAEDTAVYYCAR

SEQ ID NO: 49 - protein, 98 aa, Homo sapiens; identical to SEQ ID NO: 48

SEQ ID NO: 50 - protein, 98 aa, Homo sapiens; identical to SEQ ID NO: 48

SEQ ID NO: 51 - protein, 98 aa, Homo sapiens; identical to SEQ ID NO: 48

SEQ ID NO: 52 - protein, 99 aa, Homo sapiens
EVHLVESGGALVQPGGSLRLSCAASGFTFSYYYMSGVRQAPGKGLEWVGFIRNKANGGTTETTSVKGRFTISRDDSKSITYLQMKSLKTEDTAVYYCSR

SEQ ID NO: 53 - protein, 99 aa, Homo sapiens
EVQLVESGGGLVQPGGSLRLSCAASGFTFSYYYMSGVRQAPGKGLEWVGFIRNKANGGTTETTSVKGRFTISRDDSKSITYLQMKSLKTEDTAVYYCSR

SEQ ID NO: 54 - protein, 98 aa, Homo sapiens
EVQLLESGGGLVQPGGSLRLSCAASGFTFSSYAMSWVRQAPGKGLEWVSAISGSGGSTYYADSVKGRFTISRDNSKNTLYLQMNSLRAEDTAVYYCAK

SEQ ID NO: 55 - protein, 98 aa, Homo sapiens
EVQLLESGGGLVQPGGSLRLSCAASGFTFSSYAMSWVRQAPGKGLEWVSAISGSGGSTYYGDSVKGRFTISRDNSKNTLYLQMNSLRAEDTAVYYCAK

SEQ ID NO: 56 - protein, 98 aa, Homo sapiens
EVQLLESGGGLVQPGGSLRLSCAASGFTFSSYAMSWVRQAPGKGLEWVSVIYSGGSSTYYADSVKGRFTISRDNSKNTLYLQMNSLRAEDTAVYYCAK

SEQ ID NO: 57 - protein, 98 aa, Homo sapiens
EVQLVESGGGLVQPGGSLRLSCAASGFTFSSYAMSWVRQAPGKGLEWVSAISGSGGSTYYADSVKGRFTISRDNSKNTLYLQMNSLRAEDTAVYYCAK

SEQ ID NO: 58 - protein, 98 aa, Homo sapiens
EVQLLESGGGLVQPGGSLRLSCAASGFTFSSYAMSWVRQAPGKGLEWVSAIYSSGSSTYYADSVKGRFTISRDNSKNTLYLQMNSLRAEDTAVYYCAK

SEQ ID NO: 59 - protein, 98 aa, Homo sapiens; identical to SEQ ID NO: 54

SEQ ID NO: 60 - protein, 96 aa, Homo sapiens
EMQLVESGGGLQKPAWSPRLSCAASQFTFSSYYMNCVRQAPGNGLELVQVNPNGGSTYLIDSGKDRFNTSRDNAKNTLHLQMNSLKTEDTALYCTR

SEQ ID NO: 61 - protein, 96 aa, Homo sapiens
EMQLVESGGGLAKPAWSPRLSCAASQFTFSSYYMNCVRQAPGNGLELVQVNPNGGSTYLIDSGKDRFNTSRDNAKNTLHLQMNSLKTEDTALYCTR

SEQ ID NO: 62 - protein, 97 aa, Homo sapiens
EMQLVESGGGLAKPAWSPRLSCAASQFTFSSYYMNCVRQAPGNGLELVGQVNPNGGSTYLIDSGKDRFNTSRDNAKNTLHLQMNSLKTEDTALYCTR

SEQ ID NO: 63 - protein, 98 aa, Homo sapiens
ETQLVESGGGLAKPGRSPRLSCAASQFTFSSYYMNCVRQAPGNGLELVGQVNPNGGSTYLIDSGKDRFNTSRDNAKNTLHLQMNSLKTEDTALYYCTR

SEQ ID NO: 64 - protein, 97 aa, Homo sapiens; identical to SEQ ID NO: 62

SEQ ID NO: 65 - protein, 96 aa, Homo sapiens
EVELIEPTEDLRQPGKFLRLSCVASRFAFSSFMSPVHQSAGKGLEVIDIKDDGSQIHHADSVKGRFSISKDNAKNSLYLQMNSQRTEDMAVYGCTG

SEQ ID NO: 66 - protein, 98 aa, Homo sapiens
QVQLVESGGGVVQPGRSLRLSCAASGFTFSSYAMHWVRQAPGKGLEWVAVISYDGSNKYYADSVKGRFTISRDNSKNTLYLQMNSLRAEDTAVYYCAR

SEQ ID NO: 67 - protein, 98 aa, Homo sapiens
QVQLVESGGGVVQPGGSLRLSCAASGFTFSSYGMHWVRQAPGKGLEWVAFIRYDGSNKYYADSVKGRFTISRDNSKNTLYLQMNSLRAEDTAVYYCAK

SEQ ID NO: 68 - protein, 98 aa, Homo sapiens
QVQLVESGGGVVQPGRSLRLSCAASGFTFSSYGMHWVRQAPGKGLEWVAVISYDGSNKYYADSVKGRFTISRDNSKNTLYLQMNSLRAEDTAVYYCAR

SEQ ID NO: 69 - protein, 98 aa, Homo sapiens
QVQLVESGGGVVQPGRSLRLSCAASGFTFSSYGMHWVRQAPGKGLEWVAVISYDGSNKYYADSVKGRFTISRDNSKNTLYLQMNSLRAEGTAVYYCAR

SEQ ID NO: 70 - protein, 98 aa, Homo sapiens
QVQLVDSGGGVVQPGRSLRLSCAASAFTFSSYAMHWVRQAPGKGLEWVAVISYDGSNKYYADSVKGRFTISRDNSKNTLYLQMNSLRAEDTAVYYCAR

SEQ ID NO: 71 - protein, 98 aa, Homo sapiens
QVQLVESGGGVVQPGRSLRLSCAASGFTFSSYAMHWVRQAPGKGLEWVAVISYDGSNKYYADSVKGRFAISRDNSKNTLYLQMNSLRAEDTAVYYCAR

SEQ ID NO: 72 - protein, 98 aa, Homo sapiens
QVQLVESGGGVVQPGRSLRLSCAASGFTFSSYAMHWVRQAPGKGLEWVAVISYDGSNKYYTDSVKGRFTISRDNSKNTLYLQMNSLRAEDTAVYYCAR

SEQ ID NO: 73 - protein, 98 aa, Homo sapiens; identical to SEQ ID NO: 66

SEQ ID NO: 74 - protein, 98 aa, Homo sapiens; identical to SEQ ID NO: 68

SEQ ID NO: 75 - protein, 98 aa, Homo sapiens; identical to SEQ ID NO: 66

SEQ ID NO: 76 - protein, 98 aa, Homo sapiens
QVQLVESGGGVVQPGRSLRLSCAASGFTFSSYAMHWVRQAPGKGLEWVAVISYDGSNKYYADSVKGRFTISRDNSKNTLYLQMSSLRAEDTAVYYCAR

SEQ ID NO: 77 - protein, 98 aa, Homo sapiens; identical to SEQ ID NO: 66

SEQ ID NO: 78 - protein, 98 aa, Homo sapiens; identical to SEQ ID NO: 66

SEQ ID NO: 79 - protein, 98 aa, Homo sapiens
QVQLVESGGGVVQPGRSLRLSCAASGFTFSSYAMHWVRQAPGKGLEWVAVISYDGSNKYYADSVKGRFTISRDNSKNTLYLQMNSLRAEDTAVYYCAK

SEQ ID NO: 80 - protein, 98 aa, Homo sapiens; identical to SEQ ID NO: 66

SEQ ID NO: 81 - protein, 98 aa, Homo sapiens; identical to SEQ ID NO: 66

SEQ ID NO: 82 - protein, 98 aa, Homo sapiens; identical to SEQ ID NO: 66

SEQ ID NO: 83 - protein, 98 aa, Homo sapiens
QVQLVESGGGVVQPGRSLRLSCAASGFTFSSYGMHWVRQAPGKGLEWVAVISYDGSNKYYADSVKGRFTISRDNSKNTLYLQMNSLRAEDTAVYYCAK

SEQ ID NO: 84 - protein, 98 aa, Homo sapiens; identical to SEQ ID NO: 67

SEQ ID NO: 85 - protein, 98 aa, Homo sapiens; identical to SEQ ID NO: 68

SEQ ID NO: 86 - protein, 98 aa, Homo sapiens; identical to SEQ ID NO: 66

SEQ ID NO: 87 - protein, 95 aa, Homo sapiens
EVQLVESGEDPRQPGGSLRLSCADSGLTFSSYRNSVSQAPGKGLEVVDIQCDGSQICYASLKSKFTISKENAKNSLYLLMNSLRAAGTAVCYCMG

SEQ ID NO: 88 - protein, 98 aa, Homo sapiens
QVQLVESGGGVVQPGRSLRLSCAASGFTFSSYGMHWVRQAPGKGLEWVAVISYDGSNKYYADSVKGRFTISRDNSKNRLYLQMNSLRAEDTAVYYCAR

SEQ ID NO: 89 - protein, 98 aa, Homo sapiens; identical to SEQ ID NO: 83

SEQ ID NO: 90 - protein, 98 aa, Homo sapiens; identical to SEQ ID NO: 68

SEQ ID NO: 91 - protein, 96 aa, Homo sapiens
EVELIESIEDLRQPGKFLRLSCVASRFAFSSFMSRVHQSPGKGLEVIDIKDDGSQIHHADSVKGRFSISKDNAKNSLYLQMNSQRAEDMDVYGCTG

SEQ ID NO: 92 - protein, 94 aa, Homo sapiens
EVQLVESGEDPRQPGGSLRLSCADSGLTFSSYRSSVSQAPGKGLEVVDIQCDGSQICYASLKSKFTISKENAKNSLYLLMNSLRAEGTAVCYCM

SEQ ID NO: 93 - protein, 96 aa, Homo sapiens; identical to SEQ ID NO: 65

SEQ ID NO: 94 - protein, 94 aa, Homo sapiens
EVQLVESGEDPRQPGGSLRLSCADSGLTFSSYRNSVSQAPGKGLEVVDIQCDGSQICYASLKSKFTISKENAKNSLYLLMNSLRAAGTAVCYCM

SEQ ID NO: 95 - protein, 96 aa, Homo sapiens
EVELIESIEDLRQPGKFLRLSCVASRFAFSSFMSRVHQSPGKGLEVIDIKDDGSQIHHADSVKGRFSISKDNAKNSLYLQMNTQRAEDVAVYGYTG

SEQ ID NO: 96 - protein, 98 aa, Homo sapiens
QVQLVESGGGVVQPGRSLRLSCAASGFTFSSYGMHWVRQAPGKGLEWVAVIWYDGSNKYYADSVKGRFTISRDNSKNTLYLQMNSLRAEDTAVYYCAR

SEQ ID NO: 97 - protein, 98 aa, Homo sapiens
QVQLVESGGGVVQPGRSLRLSCAASGFTFSSYGMHWVRQAPGKGLEWVAVIWYDGSNKYYADSAKGRFTISRDNSTNTLFLQMNSLRAEDTAVYYCAR

SEQ ID NO: 98 - protein, 98 aa, Homo sapiens; identical to SEQ ID NO: 96

SEQ ID NO: 99 - protein, 98 aa, Homo sapiens; identical to SEQ ID NO: 68

SEQ ID NO: 100 - protein, 96 aa, Homo sapiens
EVQLVESGEDPRQPGGSLRLSCADSGLTFSSYMSSVSQAPGKGLEVVDIQCDGSQICYAQSVKSKFTISKENAKNSLYLQMNSLRAEGTAVCYCMG

SEQ ID NO: 101 - protein, 98 aa, Homo sapiens
QVQLVESGGGVVQPGRSLRLSCAASGFTFSSYGMHWVRQAPGKGLEWVAVIWYDGSNKYYADSVKGRFTISRDNSKNTLYLQMNSLRAEDTAVYYCAK

SEQ ID NO: 102 - protein, 98 aa, Homo sapiens; identical to SEQ ID NO: 101

SEQ ID NO: 103 - protein, 98 aa, Homo sapiens
EVQLVESGGGLVQPGGSLRLSCAASGFTFSNSDMNWVHQAPGKGLEWVSGVSWNGSRTHYADSVKGRFIISRDNSRNTLYLQTNSLRAEDTAVYYCVR

SEQ ID NO: 104 - protein, 97 aa, Homo sapiens
EVQLVESGGGLVQPRGSLRLSCAASGFTVSSNEMSWIRQAPGKGLEWVSSISGGSTYYADSRKGRFTISRDNSKNTLYLQMNNLRAEGTAAYYCARY

SEQ ID NO: 105 - protein, 97 aa, Homo sapiens
EVQLVESGGGLVQPRGSLRLSCAASGFTVSSNEMSWIRQAPGKGLEWVSSISGGSTYYADSRKGRFTISRDNSKNTLYLQMNNLRAEGTAVYYCARY

SEQ ID NO: 106 - protein, 97 aa, Homo sapiens; identical to SEQ ID NO: 105

SEQ ID NO: 107 - protein, 96 aa, Homo sapiens
EVQLVESRGVLVQPGGSLRLSCAASGFTVSSNEMSWVRQAPGKGLEWVSSISGGSTYYADSRKGRFTISRDNSKNTLHLQMNSLRAEDTAVYYCKK

SEQ ID NO: 108 - protein, 99 aa, Homo sapiens
EVQLVESGGVVVQPGGSLRLSCAASGFTFDDYTMHWVRQAPGKGLEWVSLISWDGGSTYYADSVKGRFTISRDNSKNSLYLQMNSLRTEDTALYYCAKD

SEQ ID NO: 109 - protein, 99 aa, Homo sapiens
EVQLVESGGGVVQPGGSLRLSCAASGFTFDDYAMHWVRQAPGKGLEWVSLISGDGGSTYYADSVKGRFTISRDNSKNSLYLQMNSLRTEDTALYYCAKD

SEQ ID NO: 110 - protein, 99 aa, Homo sapiens
EVQLVESGGVVVQPGGSLRLSCAASGFTFDDYAMHWVRQAPGKGLEWVSLISWDGGSTYYADSVKGRFTISRDNSKNSLYLQMNSLRAEDTALYYCAKD

SEQ ID NO: 111 - protein, 97 aa, Homo sapiens
EDQLVESGGGLVQPGGSLRPSCAASGFAFSSYALHWVRRAPGKGLEWVSAIGTGGDTYYADSVMGRFTISRDNAKKSLYLHMNSLIAEDMAVYYCAR

SEQ ID NO: 112 - protein, 97 aa, Homo sapiens
EDQLVESGGGLVQPGGSLRPSCAASGFAFSSYVLHWVRRAPGKGPEWVSAIGTGGDTYYADSVMGRFTISRDNAKKSLYLQMNSLIAEDMAVYYCAR

SEQ ID NO: 113 - protein, 98 aa, Homo sapiens
EVQLVESGGGLVQPGGSLRLSCAASGFTFSSYSMNWVRQAPGKGLEWVSYISSSSSTIYYADSVKGRFTISRDNAKNSLYLQMNSLRAEDTAVYYCAR

SEQ ID NO: 114 - protein, 98 aa, Homo sapiens
EVQLVESGGGLVQPGGSLRLSCAASGFTFSSYSMNWVRQAPGKGLEWVSYISSSSSTIYYADSVKGRFTISRDNAKNSLYLQMNSLRDEDTAVYYCAR

SEQ ID NO: 115 - protein, 98 aa, Homo sapiens
EVQLVESGGGLVQPGGSLRLSCAASGFTFSSYEMNWVRQAPGKGLEWVSYISSSGSTIYYADSVKGRFTISRDNAKNSLYLQMNSLRAEDTAVYYCAR

SEQ ID NO: 116 - protein, 98 aa, Homo sapiens; identical to SEQ ID NO: 113

SEQ ID NO: 117 - protein, 100 aa, Homo sapiens
EVQLVESGGGLVQPGRSLRLSCTASGFTFGDYAMSWFRQAPGKGLEWVGFIRSKAYGGTTEYTASVKGRFTISRDGSKSIAYLQMNSLKTEDTAVYYCTR

SEQ ID NO: 118 - protein, 100 aa, Homo sapiens
EVQLVESGGGLVQPGPSLRLSCTASGFTFGYYPMSWVRQAPGKGLEWVGFIRSKAYGGTTEYAASVKGRFTISRDDSKSIAYLQMNSLKTEDTAVYYCTR

SEQ ID NO: 119 - protein, 100 aa, Homo sapiens
EVQLVESGGGLVQPGRSLRLSCTASGFTFGDYAMSWFRQAPGKGLEWVGFIRSKAYGGTTEYAASVKGRFTISRDDSKSIAYLQMNSLKTEDTAVYYCTR

SEQ ID NO: 120 - protein, 100 aa, Homo sapiens
EVQLVESGGGLVQPGRSLRLSCTASGFTFGDYAMSWVRQAPGKGLEWVGFIRSKAYGGTTEYAASVKGRFTISRDDSKSIAYLQMNSLKTEDTAVYYCTR

SEQ ID NO: 121 - protein, 100 aa, Homo sapiens
EVQLVESGGGLVKPGRSLRLSCTASGFTFGDYAMSWFRQAPGKGLEWVGFIRSKAYGGTTEYAASVKGRFTISRDDSKSIAYLQMNSLKTEDTAVYYCTR

SEQ ID NO: 122 - protein, 97 aa, Homo sapiens
EVQLVESGGLVQPGGSLRLSCAASGFTFSSSWMHWVCQAPEKGLEWVADIKCDGSEKYYVDSVKGRLTISRDNAKNSLYLQVNSLRAEDMTVYYCVR

SEQ ID NO: 123 - protein, 97 aa, Homo sapiens
EVQLVESGGLVQPGGSLRLSCAASGFTFSSSWMHWVCQAPEKGQEWVADIKCDGSEKYYVDSVKGRLTISRDNAKNSLYLQVNSLRAEDMTVYYCVR

SEQ ID NO: 124 - protein, 97 aa, Homo sapiens; identical to SEQ ID NO: 122

SEQ ID NO: 125 - protein, 97 aa, Homo sapiens
EVQLVESGGGLIQPGGSLRLSCAASGFTVSSNYMSWVRQAPGKGLEWVSVIYSGGSTYYADSVKGRFTISRDNSKNTLYLQMNSLRAEDTAVYYCAR

SEQ ID NO: 126 - protein, 97 aa, Homo sapiens
EVQLVETGGGLIQPGGSLRLSCAASGFTVSSNYMSWVRQAPGKGLEWVSVIYSGGSTYYADSVKGRFTISRDNSKNTLYLQMNSLRAEDTAVYYCAR

SEQ ID NO: 127 - protein, 97 aa, Homo sapiens
EVQLVESGGGLIQPGGSLRLSCAASGFTVSSNYMSWVRQPPGKGLEWVSVIYSGGSTYYADSVKGRFTISRDNSKNTLYLQMNSLRAEDTAVYYCAR

SEQ ID NO: 128 - protein, 97 aa, Homo sapiens
EVQLVESGGGLVQPGGSLRLSCAASGFTVSSNYMSWVRQAPGKGLEWVSVIYSGGSTYYADSVKGRFTISRHNSKNTLYLQMNSLRAEDTAVYYCAR

SEQ ID NO: 129 - protein, 93 aa, Homo sapiens
EVQLVESEENQRQLGGSLRLSCADSGLTFSSYMSSDSQAPGKGLEVVDIDRSQLCYAQSVKSRFTISKENAKNSLCLQMNSLRAEGTAVYYCM

SEQ ID NO: 130 - protein, 94 aa, Homo sapiens
EVQLVESEENQRQLGGSLRLSCADSGLTFSSYMSSDSQAPGKGLEVVDIYDRSQICYAQSVKSRFTISKENAKNSLRLQMNSLRAEGTAVYYCM

SEQ ID NO: 131 - protein, 93 aa, Homo sapiens; identical to SEQ ID NO: 129

SEQ ID NO: 132 - protein, 97 aa, Homo sapiens
EVQLVESGEGLVQPGGSLRLSCAASGFTFSSSAMHWVRQAPRKGLWVSVISTSGDTVLYTDSVKGRFTISRDNAQNSLSLQMNSLRAEGTVVYYCVK

SEQ ID NO: 133 - protein, 97 aa, Homo sapiens
EVELIESIEGLRQLGKFLRLSCVASGFTFSSYMSWVNETLGKGLEGVIDVKYDGSQIYHADSVKGRFTISKDNAKNSPYLQTNSLRAEDMTMHGCTG

SEQ ID NO: 134 - protein, 96 aa, Homo sapiens
EVELIESIEGLRQLGKFLRLSCVASGFTFSSYMSWVNETLGKGLEGVIDVKYDGSQIYHADSVKGRFTISKDNAKNSPYLQTNSLRAEDMTMHGCT

SEQ ID NO: 135 - protein, 98 aa, Homo sapiens
EVQLVESGGGLVQPGGSLRLSCAASGFTFSSYAMHWVRQAPGKGLEYVSAISSNGGSTYYANSVKGRFTISRDNSKNTLYLQMGSLRAEDMAVYYCAR

SEQ ID NO: 136 - protein, 98 aa, Homo sapiens
EVQLVESGEGLVQPGGSLRLSCAASGFTFSSYAMHWVRQAPGKGLEYVSAISSNGGSTYYADSVKGRFTISRDNSKNTLYLQMGSLRAEDMAVYYCAR

SEQ ID NO: 137 - protein, 98 aa, Homo sapiens
EVQLVESGGGLVQPGGSLRLSCSASGFTFSSYAMHWVRQAPGKGLEYVSAISSNGGSTYYADSVKGRFTISRDNSKNTLYVQMSSLRAEDTAVYYCVK

SEQ ID NO: 138 - protein, 98 aa, Homo sapiens
QVQLVESGGGLVQPGGSLRLSCSASGFTFSSYAMHWVRQAPGKGLEYVSAISSNGGSTYYADSVKGRFTISRDNSKNTLYLQMNSLRAEDTAVYYCAR

SEQ ID NO: 139 - protein, 98 aa, Homo sapiens; identical to SEQ ID NO: 137

SEQ ID NO: 140 - protein, 98 aa, Homo sapiens
EVQLVESGGGLVQPGGSLRLSCSASGFTFSSYAMHWVRQAPGKGLEYVSAISSNGGSTYYADSVKGRFTISRDNSKNTLYLQMSSLRAEDTAVYYCVK

SEQ ID NO: 141 - protein, 97 aa, Homo sapiens
EVQLVESGGGLVQPGGSLRLSCAASGFTVSSNYMSWVRQAPGKGLEWVSVIYSGGSTYYADSVKGRFTISRDNSKNTLYLQMNSLRAEDTAVYYCAR

SEQ ID NO: 142 - protein, 97 aa, Homo sapiens; identical to SEQ ID NO: 141

SEQ ID NO: 143 - protein, 97 aa, Homo sapiens
EVQLVESGGGLIQPGGSLRLSCAASGFTVSSNYMSWVRQAPGKGLEWVSVIYSCGSTYYADSVKGRFTISRDNSKNTLYLQMNSLRAEDTAVYYCAR

SEQ ID NO: 144 - protein, 97 aa, Homo sapiens; identical to SEQ ID NO: 141

SEQ ID NO: 145 - protein, 97 aa, Homo sapiens
EVQLVESGGGLVKPGGSLRLSCAASGFTFSDYYMNWVRQAPGKGLEWVSSISSSSTIYYADSVKGRFTISRDNAKNSLYLQMNSLRAEDTAVYYCAR

SEQ ID NO: 146 - protein, 97 aa, Homo sapiens; identical to SEQ ID NO: 145

SEQ ID NO: 147 - protein, 99 aa, Homo sapiens
EVQLVESGGGLVQPGGSLRLSCAASGFTFSDYYMSWVRQAPGKGLEWVGFIRNKANGGTTETTSVKGRFTISRDDSKSITYLQMNSLRAEDTAVYYCAR

SEQ ID NO: 148 - protein, 99 aa, Homo sapiens
EVQLVESGGGLVQPGGSLRLSCAASGFTFSDYYMSWVRQAPGKGLEWVGFIRNKANGGTTETTSVKGRFTISRDDSKSITYLQMNSLRAEDMAVYYCAR

SEQ ID NO: 149 - protein, 99 aa, Homo sapiens; identical to SEQ ID NO: 147

SEQ ID NO: 150 - protein, 100 aa, Homo sapiens
EVQLVESGGGLVQPGGSLRLSCAASGFTFSDHYMDWVRQAPGKGLEWVGRTRNKANSYTTEYAASVKGRFTISRDDSKNSLYLQMNSLKTEDTAVYYCAR

SEQ ID NO: 151 - protein, 55 aa, Homo sapiens
TFSDHYMDWVRQAPGKGLEWVGRTRNKANSYTTEYAASVKGRFTISRDDSKNSLY

SEQ ID NO: 152 - protein, 100 aa, Homo sapiens
EVQLVESGGGLVQPGGSLKLSCAASGFTFSGSAMHWVRQASGKGLEWVGRIRSKANSYATAYAASVKGRFTISRDDSKNTAYLQMNSLKTEDTAVYYCTR

SEQ ID NO: 153 - protein, 100 aa, Homo sapiens; identical to SEQ ID NO: 152

SEQ ID NO: 154 - protein, 98 aa, Homo sapiens
EVQLVESGGGLVQPGGSLRLSCAASGFTFSSYWMHWVRQAPGKGLVWVSRINSDGSSTSYADSVKGRFTISRDNAKNTLYLQMNSLRAEDTAVYYCAR

SEQ ID NO: 155 - protein, 98 aa, Homo sapiens; identical to SEQ ID NO: 154

SEQ ID NO: 156 - protein, 98 aa, Homo sapiens
EVQLVESGGGLVQPGGSLRLSCAASGFTFSSYWMHWVRQAPGKGLVWVSRINSDGSSTTYADSVKGRFTISRDNAKNTLYLQMNSLRAEDTAVYYCAR

SEQ ID NO: 157 - protein, 98 aa, Homo sapiens
QVQLVESGGGVVQPGGSLRLSCAASGFTFSSYGMHWVRQAPGKGLEWVSVIYSGGSSTYYADSVKGRFTISRDNSKNTLYLQMNSLRAEDTAVYYCAK